European Patent Application EP 4 134 089 A1, published February 15, 2023. Title: Pharmaceutical composition for prevention or treatment of cancer comprising Leuconostoc sp. as active ingredient. Applicant: LISCure Biosciences Inc. The sequence listing filed with the application follows.

SEQUENCE LISTING (1 sequence)

SEQ ID NO: 1 - DNA, 1487 bp, Leuconostoc mesenteroides
tctgtcaggatgaacgctggcggcgtgcctaatacatgcaagtcgaacgcacagcgaaaggtgcttgcacctttcaagtgagtggcgaacgggtgagtaacacgtggacaacctgcctcaaggctggggataacatttggaaacagatgctaataccgaataaaacttagtgtcgcatgacacaaagttaaaaggcgcttcggcgtcacctagagatggatccgcggtgcattagttagttggtggggtaaaggcctaccaagacaatgatgcatagccgagttgagagactgatcggccacattgggactgagacacggcccaaactcctacgggaggctgcagtagggaatcttccacaatgggcgaaagcctgatggagcaacgccgcgtgtgtgatgaaggctttcgggtcgtaaagcactgttgtatgggaagaacagctagaataggaaatgattttagtttgacggtaccataccagaaagggacggctaaatacgtgccagcagccgcggtaatacgtatgtcccgagcgttatccggatttattgggcgtaaagcgagcgcagacggtttattaagtctgatgtgaaagcccggagctcaactccggaatggcattggaaactggttaacttgagtgcagtagaggtaagtggaactccatgtgtagcggtggaatgcgtagatatatggaagaacaccagtggcgaaggcggcttactggactgcaactgacgttgaggctcgaaagtgtgggtagcaaacaggattagataccctggtagtccacaccgtaaacgatgaacactaggtgttaggaggtttccgcctcttagtgccgaagctaacgcattaagtgttccgcctggggagtacgaccgcaaggttgaaactcaaaggaattgacggggacccgcacaagcggtggagcatgtggtttaattcgaagcaacgcgaagaaccttaccaggtcttgacatcctttgaagcttttagagatagaagtgttctcttcggagacaaagtgacaggtggtgcatggtcgtcgtcagctcgtgtcgtgagatgttgggttaagtcccgcaacgagcgcaacccttattgttagttgccagcattcagatgggcactctagcgagactgccggtgacaaaccggaggaaggcggggacgacgtcagatcatcatgccccttatgacctgggctacacacgtgctacaatggcgtatacaacgagttgccagcccgcgagggtgagctaatctcttaaagtacgtctcagttcggattgtagtctgcaactcgactacatgaagtcggaatcgctagtaatcgcggatcagcacgccgcggtgaatacgttcccgggtcttgtacacaccgcccgtcacaccatgggagtttgtaatgcccaaagccggtggcctaaccttttaggaaggagccgtctaaggcaggacagatgactggggtgaagtct